European Patent Specification EP 3 693 384 B1, published January 24, 2024. Title: METHOD FOR GENERATING T-CELLS COMPATIBLE FOR ALLOGENIC TRANSPLANTATION. Applicant: Cellectis. The sequence listing filed with the application follows.

SEQUENCE LISTING (97 sequences)

SEQ ID NO: 1 - protein, 119 aa, Homo sapiens
MSRSVALAVLALLSLSGLEAIQRTPKIQVYSRHPAENGKSNFLNCYVSGFHPSDIEVDLLKNGERIEKVEHSDLSFSKDWSFYLLYYTEFTPTEKDEYACRVNHVTLSQPKIVKWDRDM

SEQ ID NO: 2 - DNA, 6673 bp, Homo sapiens
aatataagtggaggcgtcgcgctggcgggcattcctgaagctgacagcattcgggccgagatgtctcgctccgtggccttagctgtgctcgcgctactctctctttctggcctggaggctatccagcgtgagtctctcctaccctcccgctctggtccttcctctcccgctctgcaccctctgtggccctcgctgtgctctctcgctccgtgacttcccttctccaagttctccttggtggcccgccgtggggctagtccagggctggatctcggggaagcggcggggtggcctgggagtggggaagggggtgcgcacccgggacgcgcgctacttgcccctttcggcggggagcaggggagacctttggcctacggcgacgggagggtcgggacaaagtttagggcgtcgataagcgtcagagcgccgaggttgggggagggtttctcttccgctctttcgcggggcctctggctcccccagcgcagctggagtgggggacgggtaggctcgtcccaaaggcgcggcgctgaggtttgtgaacgcgtggaggggcgcttggggtctgggggaggcgtcgcccgggtaagcctgtctgctgcggctctgcttcccttagactggagagctgtggacttcgtctaggcgcccgctaagttcgcatgtcctagcacctctgggtctatgtggggccacaccgtggggaggaaacagcacgcgacgtttgtagaatgcttggctgtgatacaaagcggtttcgaataattaacttatttgttcccatcacatgtcacttttaaaaaattataagaactacccgttattgacatctttctgtgtgccaaggactttatgtgctttgcgtcatttaattttgaaaacagttatcttccgccatagataactactatggttatcttctgcctctcacagatgaagaaactaaggcaccgagattttaagaaacttaattacacaggggataaatggcagcaatcgagattgaagtcaagcctaaccagggcttttgcgggagcgcatgccttttggctgtaattcgtgcatttttttttaagaaaaacgcctgccttctgcgtgagattctccagagcaaactgggcggcatgggccctgtggtcttttcgtacagagggcttcctctttggctctttgcctggttgtttccaagatgtactgtgcctcttactttcggttttgaaaacatgagggggttgggcgtggtagcttacgcctgtaatcccagcacttagggaggccgaggcgggaggatggcttgaggtccgtagttgagaccagcctggccaacatggtgaagcctggtctctacaaaaaataataacaaaaattagccgggtgtggtggctcgtgcctgtggtcccagctgctccggtggctgaggcgggaggatctcttgagcttaggcttttgagctatcatggcgccagtgcactccagcgtgggcaacagagcgagaccctgtctctcaaaaaagaaaaaaaaaaaaaaagaaagagaaaagaaaagaaagaaagaagtgaaggtttgtcagtcaggggagctgtaaaaccattaataaagataatccaagatggttaccaagactgttgaggacgccagagatcttgagcactttctaagtacctggcaatacactaagcgcgctcaccttttcctctggcaaaacatgatcgaaagcagaatgttttgatcatgagaaaattgcatttaatttgaatacaatttatttacaacataaaggataatgtatatatcaccaccattactggtatttgctggttatgttagatgtcattttaaaaaataacaatctgatatttaaaaaaaaatcttattttgaaaatttccaaagtaatacatgccatgcatagaccatttctggaagataccacaagaaacatgtaatgatgattgcctctgaaggtctattttcctcctctgacctgtgtgtgggttttgtttttgttttactgtgggcataaattaatttttcagttaagttttggaagcttaaataactctccaaaagtcataaagccagtaactggttgagcccaaattcaaacccagcctgtctgatacttgtcctcttcttagaaaagattacagtgatgctctcacaaaatcttgccgccttccctcaaacagagagttccaggcaggatgaatctgtgctctgatccctgaggcatttaatatgttcttattattagaagctcagatgcaaagagctctcttagcttttaatgttatgaaaaaaatcaggtcttcattagattccccaatccacctcttgatggggctagtagcctttccttaatgatagggtgtttctagagagatatatctggtcaaggtggcctggtactcctccttctccccacagcctcccagacaaggaggagtagctgccttttagtgatcatgtaccctgaatataagtgtatttaaaagaattttatacacatatatttagtgtcaatctgtatatttagtagcactaacacttctcttcattttcaatgaaaaatatagagtttataatattttcttcccacttccccatggatggtctagtcatgcctctcattttggaaagtactgtttctgaaacattaggcaatatattcccaacctggctagtttacagcaatcacctgtggatgctaattaaaacgcaaatcccactgtcacatgcattactccatttgatcataatggaaagtatgttctgtcccatttgccatagtcctcacctatccctgttgtattttatcgggtccaactcaaccatttaaggtatttgccagctcttgtatgcatttaggttttgtttctttgttttttagctcatgaaattaggtacaaagtcagagaggggtctggcatataaaacctcagcagaaataaagaggttttgttgtttggtaagaacataccttgggttggttgggcacggtggctcgtgcctgtaatcccaacactttgggaggccaaggcaggctgatcacttgaagttgggagttcaagaccagcctggccaacatggtgaaatcccgtctctactgaaaatacaaaaattaaccaggcatggtggtgtgtgcctgtagtcccaggaatcacttgaacccaggaggcggaggttgcagtgagctgagatctcaccactgcacactgcactccagcctgggcaatggaatgagattccatcccaaaaaataaaaaaataaaaaaataaagaacataccttgggttgatccacttaggaacctcagataataacatctgccacgtatagagcaattgctatgtcccaggcactctactagacacttcatacagtttagaaaatcagatgggtgtagatcaaggcaggagcaggaaccaaaaagaaaggcataaacataagaaaaaaaatggaaggggtggaaacagagtacaataacatgagtaatttgatgggggctattatgaactgagaaatgaactttgaaaagtatcttggggccaaatcatgtagactcttgagtgatgtgttaaggaatgctatgagtgctgagagggcatcagaagtccttgagagcctccagagaaaggctcttaaaaatgcagcgcaatctccagtgacagaagatactgctagaaatctgctagaaaaaaaacaaaaaaggcatgtatagaggaattatgagggaaagataccaagtcacggtttattcttcaaaatggaggtggcttgttgggaaggtggaagctcatttggccagagtggaaatggaattgggagaaatcgatgaccaaatgtaaacacttggtgcctgatatagcttgacaccaagttagccccaagtgaaataccctggcaatattaatgtgtcttttcccgatattcctcaggtactccaaagattcaggtttactcacgtcatccagcagagaatggaaagtcaaatttcctgaattgctatgtgtctgggtttcatccatccgacattgaagttgacttactgaagaatggagagagaattgaaaaagtggagcattcagacttgtctttcagcaaggactggtctttctatctcttgtactacactgaattcacccccactgaaaaagatgagtatgcctgccgtgtgaaccatgtgactttgtcacagcccaagatagttaagtggggtaagtcttacattcttttgtaagctgctgaaagttgtgtatgagtagtcatatcataaagctgctttgatataaaaaaggtctatggccatactaccctgaatgagtcccatcccatctgatataaacaatctgcatattgggattgtcagggaatgttcttaaagatcagattagtggcacctgctgagatactgatgcacagcatggtttctgaaccagtagtttccctgcagttgagcagggagcagcagcagcacttgcacaaatacatatacactcttaacacttcttacctactggcttcctctagcttttgtggcagcttcaggtatatttagcactgaacgaacatctcaagaaggtataggcctttgtttgtaagtcctgctgtcctagcatcctataatcctggacttctccagtactttctggctggattggtatctgaggctagtaggaagggcttgttcctgctgggtagctctaaacaatgtattcatgggtaggaacagcagcctattctgccagccttatttctaaccattttagacatttgttagtacatggtattttaaaagtaaaacttaatgtcttccttttttttctccactgtctttttcatagatcgagacatgtaagcagcatcatggaggtaagtttttgaccttgagaaaatgtttttgtttcactgtcctgaggactatttatagacagctctaacatgataaccctcactatgtggagaacattgacagagtaacattttagcagggaaagaagaatcctacagggtcatgttcccttctcctgtggagtggcatgaagaaggtgtatggccccaggtatggccatattactgaccctctacagagagggcaaaggaactgccagtatggtattgcaggataaaggcaggtggttacccacattacctgcaaggctttgatctttcttctgccatttccacattggacatctctgctgaggagagaaaatgaaccactcttttcctttgtataatgttgttttattcttcagacagaagagaggagttatacagctctgcagacatcccattcctgtatggggactgtgtttgcctcttagaggttcccaggccactagaggagataaagggaaacagattgttataacttgatataatgatactataatagatgtaactacaaggagctccagaagcaagagagagggaggaacttggacttctctgcatctttagttggagtccaaaggcttttcaatgaaattctactgcccagggtacattgatgctgaaaccccattcaaatctcctgttatattctagaacagggaattgatttgggagagcatcaggaaggtggatgatctgcccagtcacactgttagtaaattgtagagccaggacctgaactctaatatagtcatgtgttacttaatgacggggacatgttctgagaaatgcttacacaaacctaggtgttgtagcctactacacgcataggctacatggtatagcctattgctcctagactacaaacctgtacagcctgttactgtactgaatactgtgggcagttgtaacacaatggtaagtatttgtgtatctaaacatagaagttgcagtaaaaatatgctattttaatcttatgagaccactgtcatatatacagtccatcattgaccaaaacatcatatcagcattttttcttctaagattttgggagcaccaaagggatacactaacaggatatactctttataatgggtttggagaactgtctgcagctacttcttttaaaaaggtgatctacacagtagaaattagacaagtttggtaatgagatctgcaatccaaataaaataaattcattgctaacctttttcttttcttttcaggtttgaagatgccgcatttggattggatgaattccaaattctgcttgcttgctttttaatattgatatgcttatacacttacactttatgcacaaaatgtagggttataataatgttaacatggacatgatcttctttataattctactttgagtgctgtctccatgtttgatgtatctgagcaggttgctccacaggtagctctaggagggctggcaacttagaggtggggagcagagaattctcttatccaacatcaacatcttggtcagatttgaactcttcaatctcttgcactcaaagcttgttaagatagttaagcgtgcataagttaacttccaatttacatactctgcttagaatttgggggaaaatttagaaatataattgacaggattattggaaatttgttataatgaatgaaacattttgtcatataagattcatatttacttcttatacatttgataaagtaaggcatggttgtggttaatctggtttatttttgttccacaagttaaataaatcataaaacttgatgtgttatctctta

SEQ ID NO: 3 - DNA, 987 bp, Homo sapiens
aatataagtggaggcgtcgcgctggcgggcattcctgaagctgacagcattcgggccgagatgtctcgctccgtggccttagctgtgctcgcgctactctctctttctggcctggaggctatccagcgtactccaaagattcaggtttactcacgtcatccagcagagaatggaaagtcaaatttcctgaattgctatgtgtctgggtttcatccatccgacattgaagttgacttactgaagaatggagagagaattgaaaaagtggagcattcagacttgtctttcagcaaggactggtctttctatctcttgtactacactgaattcacccccactgaaaaagatgagtatgcctgccgtgtgaaccatgtgactttgtcacagcccaagatagttaagtgggatcgagacatgtaagcagcatcatggaggtttgaagatgccgcatttggattggatgaattccaaattctgcttgcttgctttttaatattgatatgcttatacacttacactttatgcacaaaatgtagggttataataatgttaacatggacatgatcttctttataattctactttgagtgctgtctccatgtttgatgtatctgagcaggttgctccacaggtagctctaggagggctggcaacttagaggtggggagcagagaattctcttatccaacatcaacatcttggtcagatttgaactcttcaatctcttgcactcaaagcttgttaagatagttaagcgtgcataagttaacttccaatttacatactctgcttagaatttgggggaaaatttagaaatataattgacaggattattggaaatttgttataatgaatgaaacattttgtcatataagattcatatttacttcttatacatttgataaagtaaggcatggttgtggttaatctggtttatttttgttccacaagttaaataaatcataaaacttgatgtgttatctctta

SEQ ID NO: 4 - protein, 1130 aa, Homo sapiens
MRCLAPRPAGSYLSEPQGSSQCATMELGPLEGGYLELLNSDADPLCLYHFYDQMDLAGEEEIELYSEPDTDTINCDQFSRLLCDMEGDEETREAYANIAELDQYVFQDSQLEGLSKDIFKHIGPDEVIGESMEMPAEVGQKSQKRPFPEELPADLKHWKPAEPPTVVTGSLLVGPVSDCSTLPCLPLPALFNQEPASGQMRLEKTDQIPMPFSSSSLSCLNLPEGPIQFVPTISTLPHGLWQISEAGTGVSSIFIYHGEVPQASQVPPPSGFTVHGLPTSPDRPGSTSPFAPSATDLPSMPEPALTSRANMTEHKTSPTQCPAAGEVSNKLPKWPEPVEQFYRSLQDTYGAEPAGPDGILVEVDLVQARLERSSSKSLERELATPDWAERQLAQGGLAEVLLAAKEHRRPRETRVIAVLGKAGQGKSYWAGAVSRAWACGRLPQYDFVFSVPCHCLNRPGDAYGLQDLLFSLGPQPLVAADEVFSHILKRPDRVLLILDGFEELEAQDGFLHSTCGPAPAEPCSLRGLLAGLFQKKLLRGCTLLLTARPRGRLVQSLSKADALFELSGFSMEQAQAYVMRYFESSGMTEHQDRALTLLRDRPLLLSHSHSPTLCRAVCQLSEALLELGEDAKLPSTLTGLYVGLLGRAALDSPPGALAELAKLAWELGRRHQSTLQEDQFPSADVRTWAMAKGLVQHPPRAAESELAFPSFLLQCFLGALWLALSGEIKDKELPQYLALTPRKKRPYDNWLEGVPRFLAGLIFQPPARCLGALLGPSAAASVDRKQKVLARYLKRLQPGTLRARQLLELLHCAHEAEEAGIWQHVVQELPGRLSFLGTRLTPPDAHVLGKALEAAGQDFSLDLRSTGICPSGLGSLVGLSCVTRFRAALSDTVALWESLQQHGETKLLQAAEEKFTIEPFKAKSLKDVEDLGKLVQTQRTRSSSEDTAGELPAVRDLKKLEFALGPVSGPQAFPKLVRILTAFSSLQHLDLDALSENKIGDEGVSQLSATFPQLKSLETLNLSQNNITDLGAYKLAEALPSLAASLLRLSLYNNCICDVGAESLARVLPDMVSLRVMDVQYNKFTAAGAQQLAASLRRCPHVETLAMWTPTIPFSVQEHLQQQDSRISLR

SEQ ID NO: 5 - DNA, 4654 bp, Homo sapiens
ggttagtgatgaggctagtgatgaggctgtgtgcttctgagctgggcatccgaaggcatccttggggaagctgagggcacgaggaggggctgccagactccgggagctgctgcctggctgggattcctacacaatgcgttgcctggctccacgccctgctgggtcctacctgtcagagccccaaggcagctcacagtgtgccaccatggagttggggcccctagaaggtggctacctggagcttcttaacagcgatgctgaccccctgtgcctctaccacttctatgaccagatggacctggctggagaagaagagattgagctctactcagaacccgacacagacaccatcaactgcgaccagttcagcaggctgttgtgtgacatggaaggtgatgaagagaccagggaggcttatgccaatatcgcggaactggaccagtatgtcttccaggactcccagctggagggcctgagcaaggacattttcaagcacataggaccagatgaagtgatcggtgagagtatggagatgccagcagaagttgggcagaaaagtcagaaaagacccttcccagaggagcttccggcagacctgaagcactggaagccagctgagccccccactgtggtgactggcagtctcctagtgggaccagtgagcgactgctccaccctgccctgcctgccactgcctgcgctgttcaaccaggagccagcctccggccagatgcgcctggagaaaaccgaccagattcccatgcctttctccagttcctcgttgagctgcctgaatctccctgagggacccatccagtttgtccccaccatctccactctgccccatgggctctggcaaatctctgaggctggaacaggggtctccagtatattcatctaccatggtgaggtgccccaggccagccaagtaccccctcccagtggattcactgtccacggcctcccaacatctccagaccggccaggctccaccagccccttcgctccatcagccactgacctgcccagcatgcctgaacctgccctgacctcccgagcaaacatgacagagcacaagacgtcccccacccaatgcccggcagctggagaggtctccaacaagcttccaaaatggcctgagccggtggagcagttctaccgctcactgcaggacacgtatggtgccgagcccgcaggcccggatggcatcctagtggaggtggatctggtgcaggccaggctggagaggagcagcagcaagagcctggagcgggaactggccaccccggactgggcagaacggcagctggcccaaggaggcctggctgaggtgctgttggctgccaaggagcaccggcggccgcgtgagacacgagtgattgctgtgctgggcaaagctggtcagggcaagagctattgggctggggcagtgagccgggcctgggcttgtggccggcttccccagtacgactttgtcttctctgtcccctgccattgcttgaaccgtccgggggatgcctatggcctgcaggatctgctcttctccctgggcccacagccactcgtggcggccgatgaggttttcagccacatcttgaagagacctgaccgcgttctgctcatcctagacggcttcgaggagctggaagcgcaagatggcttcctgcacagcacgtgcggaccggcaccggcggagccctgctccctccgggggctgctggccggccttttccagaagaagctgctccgaggttgcaccctcctcctcacagcccggccccggggccgcctggtccagagcctgagcaaggccgacgccctatttgagctgtccggcttctccatggagcaggcccaggcatacgtgatgcgctactttgagagctcagggatgacagagcaccaagacagagccctgacgctcctccgggaccggccacttcttctcagtcacagccacagccctactttgtgccgggcagtgtgccagctctcagaggccctgctggagcttggggaggacgccaagctgccctccacgctcacgggactctatgtcggcctgctgggccgtgcagccctcgacagcccccccggggccctggcagagctggccaagctggcctgggagctgggccgcagacatcaaagtaccctacaggaggaccagttcccatccgcagacgtgaggacctgggcgatggccaaaggcttagtccaacacccaccgcgggccgcagagtccgagctggccttccccagcttcctcctgcaatgcttcctgggggccctgtggctggctctgagtggcgaaatcaaggacaaggagctcccgcagtacctagcattgaccccaaggaagaagaggccctatgacaactggctggagggcgtgccacgctttctggctgggctgatcttccagcctcccgcccgctgcctgggagccctactcgggccatcggcggctgcctcggtggacaggaagcagaaggtgcttgcgaggtacctgaagcggctgcagccggggacactgcgggcgcggcagctgctggagctgctgcactgcgcccacgaggccgaggaggctggaatttggcagcacgtggtacaggagctccccggccgcctctcttttctgggcacccgcctcacgcctcctgatgcacatgtactgggcaaggccttggaggcggcgggccaagacttctccctggacctccgcagcactggcatttgcccctctggattggggagcctcgtgggactcagctgtgtcacccgtttcagggctgccttgagcgacacggtggcgctgtgggagtccctgcagcagcatggggagaccaagctacttcaggcagcagaggagaagttcaccatcgagcctttcaaagccaagtccctgaaggatgtggaagacctgggaaagcttgtgcagactcagaggacgagaagttcctcggaagacacagctggggagctccctgctgttcgggacctaaagaaactggagtttgcgctgggccctgtctcaggcccccaggctttccccaaactggtgcggatcctcacggccttttcctccctgcagcatctggacctggatgcgctgagtgagaacaagatcggggacgagggtgtctcgcagctctcagccaccttcccccagctgaagtccttggaaaccctcaatctgtcccagaacaacatcactgacctgggtgcctacaaactcgccgaggccctgccttcgctcgctgcatccctgctcaggctaagcttgtacaataactgcatctgcgacgtgggagccgagagcttggctcgtgtgcttccggacatggtgtccctccgggtgatggacgtccagtacaacaagttcacggctgccggggcccagcagctcgctgccagccttcggaggtgtcctcatgtggagacgctggcgatgtggacgcccaccatcccattcagtgtccaggaacacctgcaacaacaggattcacggatcagcctgagatgatcccagctgtgctctggacaggcatgttctctgaggacactaaccacgctggaccttgaactgggtacttgtggacacagctcttctccaggctgtatcccatgagcctcagcatcctggcacccggcccctgctggttcagggttggcccctgcccggctgcggaatgaaccacatcttgctctgctgacagacacaggcccggctccaggctcctttagcgcccagttgggtggatgcctggtggcagctgcggtccacccaggagccccgaggccttctctgaaggacattgcggacagccacggccaggccagagggagtgacagaggcagccccattctgcctgcccaggcccctgccaccctggggagaaagtacttctttttttttatttttagacagagtctcactgttgcccaggctggcgtgcagtggtgcgatctgggttcactgcaacctccgcctcttgggttcaagcgattcttctgcttcagcctcccgagtagctgggactacaggcacccaccatcatgtctggctaatttttcatttttagtagagacagggttttgccatgttggccaggctggtctcaaactcttgacctcaggtgatccacccacctcagcctcccaaagtgctgggattacaagcgtgagccactgcaccgggccacagagaaagtacttctccaccctgctctccgaccagacaccttgacagggcacaccgggcactcagaagacactgatgggcaacccccagcctgctaattccccagattgcaacaggctgggcttcagtggcagctgcttttgtctatgggactcaatgcactgacattgttggccaaagccaaagctaggcctggccagatgcaccagcccttagcagggaaacagctaatgggacactaatggggcggtgagaggggaacagactggaagcacagcttcatttcctgtgtcttttttcactacattataaatgtctctttaatgtcacaggcaggtccagggtttgagttcataccctgttaccattttggggtacccactgctctggttatctaatatgtaacaagccaccccaaatcatagtggcttaaaacaacactcacattta

SEQ ID NO: 6 - protein, 495 aa, Artificial Sequence
  anti-CD19 Cimeric Antigen Receptor
METDTLLLWVLLLWVPGSTGEVQLQQSGPELIKPGASVKMSCKASGYTFTSYVMHWVKQKPGQGLEWIGYINPYNDGTKYNEKFKGKATLTSDKSSSTAYMELSSLTSEDSAVYYCARGTYYYGSRVFDYWGQGTTLTVSSGGGGSGGGGSGGGGSDIVMTQAAPSIPVTPGESVSISCRSSKSLLNSNGNTYLYWFLQRPGQSPQLLIYRMSNLASGVPDRFSGSGSGTAFTLRISRVEAEDVGVYYCMQHLEYPFTFGAGTKLELKRSDPTTTPAPRPPTPAPTIASQPLSLRPEACRPAAGGAVHTRGLDFACDIYIWAPLAGTCGVLLLSLVITLYCKRGRKKLLYIFKQPFMRPVQTTQEEDGCSCRFPEEEEGGCELRVKFSRSADAPAYQQGQNQLYNELNLGRREEYDVLDKRRGRDPEMGGKPRRKNPQEGLYNELQKDKMAEAYSEIGMKGERRRGKGHDGLYQGLSTATKDTYDALHMQALPPR

SEQ ID NO: 7 - protein, 17 aa, Artificial Sequence
  ANti-CD19 CAR
AAAAAAAAAAAAAAAAA

SEQ ID NO: 8 - DNA, 23 bp, Homo sapiens
gagaatcaaaatcggtgaatagg

SEQ ID NO: 9 - DNA, 23 bp, Homo sapiens
ttcaaaacctgtcagtgattggg

SEQ ID NO: 10 - DNA, 23 bp, Homo sapiens
tgtgctagacatgaggtctatgg

SEQ ID NO: 11 - DNA, 23 bp, Homo sapiens
cgtcatgagcagattaaacccgg

SEQ ID NO: 12 - DNA, 23 bp, Homo sapiens
tcagggttctggatatctgtggg

SEQ ID NO: 13 - DNA, 23 bp, Homo sapiens
gtcagggttctggatatctgtgg

SEQ ID NO: 14 - DNA, 23 bp, Homo sapiens
ttcggaacccaatcactgacagg

SEQ ID NO: 15 - DNA, 23 bp, Homo sapiens
taaacccggccactttcaggagg

SEQ ID NO: 16 - DNA, 23 bp, Homo sapiens
aaagtcagatttgttgctccagg

SEQ ID NO: 17 - DNA, 23 bp, Homo sapiens
aacaaatgtgtcacaaagtaagg

SEQ ID NO: 18 - DNA, 23 bp, Homo sapiens
tggatttagagtctctcagctgg

SEQ ID NO: 19 - DNA, 23 bp, Homo sapiens
taggcagacagacttgtcactgg

SEQ ID NO: 20 - DNA, 23 bp, Homo sapiens
agctggtacacggcagggtcagg

SEQ ID NO: 21 - DNA, 23 bp, Homo sapiens
gctggtacacggcagggtcaggg

SEQ ID NO: 22 - DNA, 23 bp, Homo sapiens
tctctcagctggtacacggcagg

SEQ ID NO: 23 - DNA, 23 bp, Homo sapiens
tttcaaaacctgtcagtgattgg

SEQ ID NO: 24 - DNA, 23 bp, Homo sapiens
gattaaacccggccactttcagg

SEQ ID NO: 25 - DNA, 23 bp, Homo sapiens
ctcgaccagcttgacatcacagg

SEQ ID NO: 26 - DNA, 23 bp, Homo sapiens
agagtctctcagctggtacacgg

SEQ ID NO: 27 - DNA, 23 bp, Homo sapiens
ctctcagctggtacacggcaggg

SEQ ID NO: 28 - DNA, 23 bp, Homo sapiens
aagttcctgtgatgtcaagctgg

SEQ ID NO: 29 - DNA, 23 bp, Homo sapiens
atcctcctcctgaaagtggccgg

SEQ ID NO: 30 - DNA, 23 bp, Homo sapiens
tgctcatgacgctgcggctgtgg

SEQ ID NO: 31 - DNA, 23 bp, Homo sapiens
acaaaactgtgctagacatgagg

SEQ ID NO: 32 - DNA, 23 bp, Homo sapiens
atttgtttgagaatcaaaatcgg

SEQ ID NO: 33 - DNA, 23 bp, Homo sapiens
catcacaggaactttctaaaagg

SEQ ID NO: 34 - DNA, 23 bp, Homo sapiens
gtcgagaaaagctttgaaacagg

SEQ ID NO: 35 - DNA, 23 bp, Homo sapiens
ccactttcaggaggaggattcgg

SEQ ID NO: 36 - DNA, 23 bp, Homo sapiens
ctgacaggttttgaaagtttagg

SEQ ID NO: 37 - DNA, 23 bp, Homo sapiens
agctttgaaacaggtaagacagg

SEQ ID NO: 38 - DNA, 23 bp, Homo sapiens
tggaataatgctgttgttgaagg

SEQ ID NO: 39 - DNA, 23 bp, Homo sapiens
agagcaacagtgctgtggcctgg

SEQ ID NO: 40 - DNA, 23 bp, Homo sapiens
ctgtggtccagctgaggtgaggg

SEQ ID NO: 41 - DNA, 23 bp, Homo sapiens
ctgcggctgtggtccagctgagg

SEQ ID NO: 42 - DNA, 23 bp, Homo sapiens
tgtggtccagctgaggtgagggg

SEQ ID NO: 43 - DNA, 23 bp, Homo sapiens
cttcttccccagcccaggtaagg

SEQ ID NO: 44 - DNA, 23 bp, Homo sapiens
acacggcagggtcagggttctgg

SEQ ID NO: 45 - DNA, 23 bp, Homo sapiens
cttcaagagcaacagtgctgtgg

SEQ ID NO: 46 - DNA, 23 bp, Homo sapiens
ctggggaagaaggtgtcttctgg

SEQ ID NO: 47 - DNA, 23 bp, Homo sapiens
tcctcctcctgaaagtggccggg

SEQ ID NO: 48 - DNA, 23 bp, Homo sapiens
ttaatctgctcatgacgctgcgg

SEQ ID NO: 49 - DNA, 23 bp, Homo sapiens
acccggccactttcaggaggagg

SEQ ID NO: 50 - DNA, 23 bp, Homo sapiens
ttcttccccagcccaggtaaggg

SEQ ID NO: 51 - DNA, 23 bp, Homo sapiens
cttacctgggctggggaagaagg

SEQ ID NO: 52 - DNA, 23 bp, Homo sapiens
gacaccttcttccccagcccagg

SEQ ID NO: 53 - DNA, 23 bp, Homo sapiens
gctgtggtccagctgaggtgagg

SEQ ID NO: 54 - DNA, 23 bp, Homo sapiens
ccgaatcctcctcctgaaagtgg

SEQ ID NO: 55 - DNA, 49 bp, Homo sapiens
ttccctcccaggcagctcacagtgtgccaccatggagttggggccccta

SEQ ID NO: 56 - DNA, 49 bp, Homo sapiens
tgcctctaccacttctatgaccagatggacctggctggagaagaagaga

SEQ ID NO: 57 - DNA, 49 bp, Homo sapiens
tcttcatccaagggacttttcctcccagaacccgacacagacaccatca

SEQ ID NO: 58 - DNA, 49 bp, Homo sapiens
tgttgtgtgacatggaaggtgatgaagagaccagggaggcttatgccaa

SEQ ID NO: 59 - DNA, 47 bp, Homo sapiens
ccaaagattcaggtttactcacgtcatccagcagagaatggaaagtc

SEQ ID NO: 60 - DNA, 49 bp, Homo sapiens
ttgtcccacagatatccagaaccctgaccctgccgtgtaccagctgaga

SEQ ID NO: 61 - DNA, 49 bp, Homo sapiens
tgtgtttgagccatcagaagcagagatctcccacacccaaaaggccaca

SEQ ID NO: 62 - DNA, 50 bp, Homo sapiens
ttcccacccgaggtcgctgtgtttgagccatcagaagcagagatctccca

SEQ ID NO: 63 - DNA, 49 bp, Homo sapiens
tttagaaagttcctgtgatgtcaagctggtcgagaaaagctttgaaaca

SEQ ID NO: 64 - DNA, 49 bp, Homo sapiens
tccagtgacaagtctgtctgcctattcaccgattttgattctcaaacaa

SEQ ID NO: 65 - DNA, 49 bp, Homo sapiens
tatatcacagacaaaactgtgctagacatgaggtctatggacttcaaga

SEQ ID NO: 66 - DNA, 49 bp, Homo sapiens
tgaggtctatggacttcaagagcaacagtgctgtggcctggagcaacaa

SEQ ID NO: 67 - DNA, 2814 bp, Artificial Sequence
  TALE-nuclease sequence
atgggcgatcctaaaaagaaacgtaaggtcatcgattacccatacgatgttccagattacgctatcgatatcgccgatctacgcacgctcggctacagccagcagcaacaggagaagatcaaaccgaaggttcgttcgacagtggcgcagcaccacgaggcactggtcggccacgggtttacacacgcgcacatcgttgcgttaagccaacacccggcagcgttagggaccgtcgctgtcaagtatcaggacatgatcgcagcgttgccagaggcgacacacgaagcgatcgttggcgtcggcaaacagtggtccggcgcacgcgctctggaggccttgctcacggtggcgggagagttgagaggtccaccgttacagttggacacaggccaacttctcaagattgcaaaacgtggcggcgtgaccgcagtggaggcagtgcatgcatggcgcaatgcactgacgggtgccccgctcaacttgaccccggagcaggtggtggccatcgccagccacgatggcggcaagcaggcgctggagacggtccagcggctgttgccggtgctgtgccaggcccacggcttgaccccggagcaggtggtggccatcgccagccacgatggcggcaagcaggcgctggagacggtccagcggctgttgccggtgctgtgccaggcccacggcttgaccccggagcaggtggtggccatcgccagcaatattggtggcaagcaggcgctggagacggtgcaggcgctgttgccggtgctgtgccaggcccacggcttgaccccggagcaggtggtggccatcgccagcaatattggtggcaagcaggcgctggagacggtgcaggcgctgttgccggtgctgtgccaggcccacggcttgaccccggagcaggtggtggccatcgccagcaatattggtggcaagcaggcgctggagacggtgcaggcgctgttgccggtgctgtgccaggcccacggcttgaccccccagcaggtggtggccatcgccagcaataatggtggcaagcaggcgctggagacggtccagcggctgttgccggtgctgtgccaggcccacggcttgaccccggagcaggtggtggccatcgccagcaatattggtggcaagcaggcgctggagacggtgcaggcgctgttgccggtgctgtgccaggcccacggcttgaccccccagcaggtggtggccatcgccagcaatggcggtggcaagcaggcgctggagacggtccagcggctgttgccggtgctgtgccaggcccacggcttgaccccccagcaggtggtggccatcgccagcaatggcggtggcaagcaggcgctggagacggtccagcggctgttgccggtgctgtgccaggcccacggcttgaccccggagcaggtggtggccatcgccagccacgatggcggcaagcaggcgctggagacggtccagcggctgttgccggtgctgtgccaggcccacggcttgaccccggagcaggtggtggccatcgccagcaatattggtggcaagcaggcgctggagacggtgcaggcgctgttgccggtgctgtgccaggcccacggcttgaccccccagcaggtggtggccatcgccagcaataatggtggcaagcaggcgctggagacggtccagcggctgttgccggtgctgtgccaggcccacggcttgaccccccagcaggtggtggccatcgccagcaataatggtggcaagcaggcgctggagacggtccagcggctgttgccggtgctgtgccaggcccacggcttgaccccccagcaggtggtggccatcgccagcaatggcggtggcaagcaggcgctggagacggtccagcggctgttgccggtgctgtgccaggcccacggcttgaccccccagcaggtggtggccatcgccagcaatggcggtggcaagcaggcgctggagacggtccagcggctgttgccggtgctgtgccaggcccacggcttgacccctcagcaggtggtggccatcgccagcaatggcggcggcaggccggcgctggagagcattgttgcccagttatctcgccctgatccggcgttggccgcgttgaccaacgaccacctcgtcgccttggcctgcctcggcgggcgtcctgcgctggatgcagtgaaaaagggattgggggatcctatcagccgttcccagctggtgaagtccgagctggaggagaagaaatccgagttgaggcacaagctgaagtacgtgccccacgagtacatcgagctgatcgagatcgcccggaacagcacccaggaccgtatcctggagatgaaggtgatggagttcttcatgaaggtgtacggctacaggggcaagcacctgggcggctccaggaagcccgacggcgccatctacaccgtgggctcccccatcgactacggcgtgatcgtggacaccaaggcctactccggcggctacaacctgcccatcggccaggccgacgaaatgcagaggtacgtggaggagaaccagaccaggaacaagcacatcaaccccaacgagtggtggaaggtgtacccctccagcgtgaccgagttcaagttcctgttcgtgtccggccacttcaagggcaactacaaggcccagctgaccaggctgaaccacatcaccaactgcaacggcgccgtgctgtccgtggaggagctcctgatcggcggcgagatgatcaaggccggcaccctgaccctggaggaggtgaggaggaagttcaacaacggcgagatcaacttcgcggccgactgataa

SEQ ID NO: 68 - DNA, 2832 bp, Artificial Sequence
  TALE-nuclease sequence
atgggcgatcctaaaaagaaacgtaaggtcatcgataaggagaccgccgctgccaagttcgagagacagcacatggacagcatcgatatcgccgatctacgcacgctcggctacagccagcagcaacaggagaagatcaaaccgaaggttcgttcgacagtggcgcagcaccacgaggcactggtcggccacgggtttacacacgcgcacatcgttgcgttaagccaacacccggcagcgttagggaccgtcgctgtcaagtatcaggacatgatcgcagcgttgccagaggcgacacacgaagcgatcgttggcgtcggcaaacagtggtccggcgcacgcgctctggaggccttgctcacggtggcgggagagttgagaggtccaccgttacagttggacacaggccaacttctcaagattgcaaaacgtggcggcgtgaccgcagtggaggcagtgcatgcatggcgcaatgcactgacgggtgccccgctcaacttgaccccccagcaggtggtggccatcgccagcaataatggtggcaagcaggcgctggagacggtccagcggctgttgccggtgctgtgccaggcccacggcttgaccccggagcaggtggtggccatcgccagcaatattggtggcaagcaggcgctggagacggtgcaggcgctgttgccggtgctgtgccaggcccacggcttgaccccggagcaggtggtggccatcgccagccacgatggcggcaagcaggcgctggagacggtccagcggctgttgccggtgctgtgccaggcccacggcttgaccccccagcaggtggtggccatcgccagcaatggcggtggcaagcaggcgctggagacggtccagcggctgttgccggtgctgtgccaggcccacggcttgaccccccagcaggtggtggccatcgccagcaatggcggtggcaagcaggcgctggagacggtccagcggctgttgccggtgctgtgccaggcccacggcttgaccccccagcaggtggtggccatcgccagcaatggcggtggcaagcaggcgctggagacggtccagcggctgttgccggtgctgtgccaggcccacggcttgaccccggagcaggtggtggccatcgccagccacgatggcggcaagcaggcgctggagacggtccagcggctgttgccggtgctgtgccaggcccacggcttgaccccggagcaggtggtggccatcgccagccacgatggcggcaagcaggcgctggagacggtccagcggctgttgccggtgctgtgccaggcccacggcttgaccccggagcaggtggtggccatcgccagcaatattggtggcaagcaggcgctggagacggtgcaggcgctgttgccggtgctgtgccaggcccacggcttgaccccccagcaggtggtggccatcgccagcaatggcggtggcaagcaggcgctggagacggtccagcggctgttgccggtgctgtgccaggcccacggcttgaccccccagcaggtggtggccatcgccagcaatggcggtggcaagcaggcgctggagacggtccagcggctgttgccggtgctgtgccaggcccacggcttgaccccggagcaggtggtggccatcgccagccacgatggcggcaagcaggcgctggagacggtccagcggctgttgccggtgctgtgccaggcccacggcttgaccccccagcaggtggtggccatcgccagcaatggcggtggcaagcaggcgctggagacggtccagcggctgttgccggtgctgtgccaggcccacggcttgaccccggagcaggtggtggccatcgccagccacgatggcggcaagcaggcgctggagacggtccagcggctgttgccggtgctgtgccaggcccacggcttgaccccccagcaggtggtggccatcgccagcaatggcggtggcaagcaggcgctggagacggtccagcggctgttgccggtgctgtgccaggcccacggcttgacccctcagcaggtggtggccatcgccagcaatggcggcggcaggccggcgctggagagcattgttgcccagttatctcgccctgatccggcgttggccgcgttgaccaacgaccacctcgtcgccttggcctgcctcggcgggcgtcctgcgctggatgcagtgaaaaagggattgggggatcctatcagccgttcccagctggtgaagtccgagctggaggagaagaaatccgagttgaggcacaagctgaagtacgtgccccacgagtacatcgagctgatcgagatcgcccggaacagcacccaggaccgtatcctggagatgaaggtgatggagttcttcatgaaggtgtacggctacaggggcaagcacctgggcggctccaggaagcccgacggcgccatctacaccgtgggctcccccatcgactacggcgtgatcgtggacaccaaggcctactccggcggctacaacctgcccatcggccaggccgacgaaatgcagaggtacgtggaggagaaccagaccaggaacaagcacatcaaccccaacgagtggtggaaggtgtacccctccagcgtgaccgagttcaagttcctgttcgtgtccggccacttcaagggcaactacaaggcccagctgaccaggctgaaccacatcaccaactgcaacggcgccgtgctgtccgtggaggagctcctgatcggcggcgagatgatcaaggccggcaccctgaccctggaggaggtgaggaggaagttcaacaacggcgagatcaacttcgcggccgactgataa

SEQ ID NO: 69 - DNA, 2814 bp, Artificial Sequence
  TALE-nuclease sequence
atgggcgatcctaaaaagaaacgtaaggtcatcgattacccatacgatgttccagattacgctatcgatatcgccgatctacgcacgctcggctacagccagcagcaacaggagaagatcaaaccgaaggttcgttcgacagtggcgcagcaccacgaggcactggtcggccacgggtttacacacgcgcacatcgttgcgttaagccaacacccggcagcgttagggaccgtcgctgtcaagtatcaggacatgatcgcagcgttgccagaggcgacacacgaagcgatcgttggcgtcggcaaacagtggtccggcgcacgcgctctggaggccttgctcacggtggcgggagagttgagaggtccaccgttacagttggacacaggccaacttctcaagattgcaaaacgtggcggcgtgaccgcagtggaggcagtgcatgcatggcgcaatgcactgacgggtgccccgctcaacttgaccccccagcaggtggtggccatcgccagcaatggcggtggcaagcaggcgctggagacggtccagcggctgttgccggtgctgtgccaggcccacggcttgaccccccagcaggtggtggccatcgccagcaataatggtggcaagcaggcgctggagacggtccagcggctgttgccggtgctgtgccaggcccacggcttgaccccccagcaggtggtggccatcgccagcaatggcggtggcaagcaggcgctggagacggtccagcggctgttgccggtgctgtgccaggcccacggcttgaccccggagcaggtggtggccatcgccagccacgatggcggcaagcaggcgctggagacggtccagcggctgttgccggtgctgtgccaggcccacggcttgaccccggagcaggtggtggccatcgccagccacgatggcggcaagcaggcgctggagacggtccagcggctgttgccggtgctgtgccaggcccacggcttgaccccggagcaggtggtggccatcgccagccacgatggcggcaagcaggcgctggagacggtccagcggctgttgccggtgctgtgccaggcccacggcttgaccccggagcaggtggtggccatcgccagcaatattggtggcaagcaggcgctggagacggtgcaggcgctgttgccggtgctgtgccaggcccacggcttgaccccggagcaggtggtggccatcgccagccacgatggcggcaagcaggcgctggagacggtccagcggctgttgccggtgctgtgccaggcccacggcttgaccccggagcaggtggtggccatcgccagcaatattggtggcaagcaggcgctggagacggtgcaggcgctgttgccggtgctgtgccaggcccacggcttgaccccccagcaggtggtggccatcgccagcaataatggtggcaagcaggcgctggagacggtccagcggctgttgccggtgctgtgccaggcccacggcttgaccccggagcaggtggtggccatcgccagcaatattggtggcaagcaggcgctggagacggtgcaggcgctgttgccggtgctgtgccaggcccacggcttgaccccccagcaggtggtggccatcgccagcaatggcggtggcaagcaggcgctggagacggtccagcggctgttgccggtgctgtgccaggcccacggcttgaccccggagcaggtggtggccatcgccagcaatattggtggcaagcaggcgctggagacggtgcaggcgctgttgccggtgctgtgccaggcccacggcttgaccccccagcaggtggtggccatcgccagcaatggcggtggcaagcaggcgctggagacggtccagcggctgttgccggtgctgtgccaggcccacggcttgaccccggagcaggtggtggccatcgccagccacgatggcggcaagcaggcgctggagacggtccagcggctgttgccggtgctgtgccaggcccacggcttgacccctcagcaggtggtggccatcgccagcaatggcggcggcaggccggcgctggagagcattgttgcccagttatctcgccctgatccggcgttggccgcgttgaccaacgaccacctcgtcgccttggcctgcctcggcgggcgtcctgcgctggatgcagtgaaaaagggattgggggatcctatcagccgttcccagctggtgaagtccgagctggaggagaagaaatccgagttgaggcacaagctgaagtacgtgccccacgagtacatcgagctgatcgagatcgcccggaacagcacccaggaccgtatcctggagatgaaggtgatggagttcttcatgaaggtgtacggctacaggggcaagcacctgggcggctccaggaagcccgacggcgccatctacaccgtgggctcccccatcgactacggcgtgatcgtggacaccaaggcctactccggcggctacaacctgcccatcggccaggccgacgaaatgcagaggtacgtggaggagaaccagaccaggaacaagcacatcaaccccaacgagtggtggaaggtgtacccctccagcgtgaccgagttcaagttcctgttcgtgtccggccacttcaagggcaactacaaggcccagctgaccaggctgaaccacatcaccaactgcaacggcgccgtgctgtccgtggaggagctcctgatcggcggcgagatgatcaaggccggcaccctgaccctggaggaggtgaggaggaagttcaacaacggcgagatcaacttcgcggccgactgataa

SEQ ID NO: 70 - DNA, 2832 bp, Artificial Sequence
  TALE-nuclease sequence
atgggcgatcctaaaaagaaacgtaaggtcatcgataaggagaccgccgctgccaagttcgagagacagcacatggacagcatcgatatcgccgatctacgcacgctcggctacagccagcagcaacaggagaagatcaaaccgaaggttcgttcgacagtggcgcagcaccacgaggcactggtcggccacgggtttacacacgcgcacatcgttgcgttaagccaacacccggcagcgttagggaccgtcgctgtcaagtatcaggacatgatcgcagcgttgccagaggcgacacacgaagcgatcgttggcgtcggcaaacagtggtccggcgcacgcgctctggaggccttgctcacggtggcgggagagttgagaggtccaccgttacagttggacacaggccaacttctcaagattgcaaaacgtggcggcgtgaccgcagtggaggcagtgcatgcatggcgcaatgcactgacgggtgccccgctcaacttgaccccggagcaggtggtggccatcgccagccacgatggcggcaagcaggcgctggagacggtccagcggctgttgccggtgctgtgccaggcccacggcttgaccccccagcaggtggtggccatcgccagcaatggcggtggcaagcaggcgctggagacggtccagcggctgttgccggtgctgtgccaggcccacggcttgaccccggagcaggtggtggccatcgccagccacgatggcggcaagcaggcgctggagacggtccagcggctgttgccggtgctgtgccaggcccacggcttgaccccggagcaggtggtggccatcgccagcaatattggtggcaagcaggcgctggagacggtgcaggcgctgttgccggtgctgtgccaggcccacggcttgaccccccagcaggtggtggccatcgccagcaataatggtggcaagcaggcgctggagacggtccagcggctgttgccggtgctgtgccaggcccacggcttgaccccggagcaggtggtggccatcgccagccacgatggcggcaagcaggcgctggagacggtccagcggctgttgccggtgctgtgccaggcccacggcttgaccccccagcaggtggtggccatcgccagcaatggcggtggcaagcaggcgctggagacggtccagcggctgttgccggtgctgtgccaggcccacggcttgaccccccagcaggtggtggccatcgccagcaataatggtggcaagcaggcgctggagacggtccagcggctgttgccggtgctgtgccaggcccacggcttgaccccccagcaggtggtggccatcgccagcaataatggtggcaagcaggcgctggagacggtccagcggctgttgccggtgctgtgccaggcccacggcttgaccccccagcaggtggtggccatcgccagcaatggcggtggcaagcaggcgctggagacggtccagcggctgttgccggtgctgtgccaggcccacggcttgaccccggagcaggtggtggccatcgccagcaatattggtggcaagcaggcgctggagacggtgcaggcgctgttgccggtgctgtgccaggcccacggcttgaccccggagcaggtggtggccatcgccagccacgatggcggcaagcaggcgctggagacggtccagcggctgttgccggtgctgtgccaggcccacggcttgaccccggagcaggtggtggccatcgccagcaatattggtggcaagcaggcgctggagacggtgcaggcgctgttgccggtgctgtgccaggcccacggcttgaccccggagcaggtggtggccatcgccagccacgatggcggcaagcaggcgctggagacggtccagcggctgttgccggtgctgtgccaggcccacggcttgaccccccagcaggtggtggccatcgccagcaataatggtggcaagcaggcgctggagacggtccagcggctgttgccggtgctgtgccaggcccacggcttgacccctcagcaggtggtggccatcgccagcaatggcggcggcaggccggcgctggagagcattgttgcccagttatctcgccctgatccggcgttggccgcgttgaccaacgaccacctcgtcgccttggcctgcctcggcgggcgtcctgcgctggatgcagtgaaaaagggattgggggatcctatcagccgttcccagctggtgaagtccgagctggaggagaagaaatccgagttgaggcacaagctgaagtacgtgccccacgagtacatcgagctgatcgagatcgcccggaacagcacccaggaccgtatcctggagatgaaggtgatggagttcttcatgaaggtgtacggctacaggggcaagcacctgggcggctccaggaagcccgacggcgccatctacaccgtgggctcccccatcgactacggcgtgatcgtggacaccaaggcctactccggcggctacaacctgcccatcggccaggccgacgaaatgcagaggtacgtggaggagaaccagaccaggaacaagcacatcaaccccaacgagtggtggaaggtgtacccctccagcgtgaccgagttcaagttcctgttcgtgtccggccacttcaagggcaactacaaggcccagctgaccaggctgaaccacatcaccaactgcaacggcgccgtgctgtccgtggaggagctcctgatcggcggcgagatgatcaaggccggcaccctgaccctggaggaggtgaggaggaagttcaacaacggcgagatcaacttcgcggccgactgataa

SEQ ID NO: 71 - DNA, 2814 bp, Artificial Sequence
  TALE-nuclease sequence
atgggcgatcctaaaaagaaacgtaaggtcatcgattacccatacgatgttccagattacgctatcgatatcgccgatctacgcacgctcggctacagccagcagcaacaggagaagatcaaaccgaaggttcgttcgacagtggcgcagcaccacgaggcactggtcggccacgggtttacacacgcgcacatcgttgcgttaagccaacacccggcagcgttagggaccgtcgctgtcaagtatcaggacatgatcgcagcgttgccagaggcgacacacgaagcgatcgttggcgtcggcaaacagtggtccggcgcacgcgctctggaggccttgctcacggtggcgggagagttgagaggtccaccgttacagttggacacaggccaacttctcaagattgcaaaacgtggcggcgtgaccgcagtggaggcagtgcatgcatggcgcaatgcactgacgggtgccccgctcaacttgaccccccagcaggtggtggccatcgccagcaataatggtggcaagcaggcgctggagacggtccagcggctgttgccggtgctgtgccaggcccacggcttgaccccccagcaggtggtggccatcgccagcaatggcggtggcaagcaggcgctggagacggtccagcggctgttgccggtgctgtgccaggcccacggcttgaccccccagcaggtggtggccatcgccagcaataatggtggcaagcaggcgctggagacggtccagcggctgttgccggtgctgtgccaggcccacggcttgaccccccagcaggtggtggccatcgccagcaatggcggtggcaagcaggcgctggagacggtccagcggctgttgccggtgctgtgccaggcccacggcttgaccccccagcaggtggtggccatcgccagcaatggcggtggcaagcaggcgctggagacggtccagcggctgttgccggtgctgtgccaggcccacggcttgaccccccagcaggtggtggccatcgccagcaatggcggtggcaagcaggcgctggagacggtccagcggctgttgccggtgctgtgccaggcccacggcttgaccccccagcaggtggtggccatcgccagcaataatggtggcaagcaggcgctggagacggtccagcggctgttgccggtgctgtgccaggcccacggcttgaccccggagcaggtggtggccatcgccagcaatattggtggcaagcaggcgctggagacggtgcaggcgctgttgccggtgctgtgccaggcccacggcttgaccccccagcaggtggtggccatcgccagcaataatggtggcaagcaggcgctggagacggtccagcggctgttgccggtgctgtgccaggcccacggcttgaccccggagcaggtggtggccatcgccagccacgatggcggcaagcaggcgctggagacggtccagcggctgttgccggtgctgtgccaggcccacggcttgaccccggagcaggtggtggccatcgccagccacgatggcggcaagcaggcgctggagacggtccagcggctgttgccggtgctgtgccaggcccacggcttgaccccggagcaggtggtggccatcgccagcaatattggtggcaagcaggcgctggagacggtgcaggcgctgttgccggtgctgtgccaggcccacggcttgaccccccagcaggtggtggccatcgccagcaatggcggtggcaagcaggcgctggagacggtccagcggctgttgccggtgctgtgccaggcccacggcttgaccccggagcaggtggtggccatcgccagccacgatggcggcaagcaggcgctggagacggtccagcggctgttgccggtgctgtgccaggcccacggcttgaccccggagcaggtggtggccatcgccagcaatattggtggcaagcaggcgctggagacggtgcaggcgctgttgccggtgctgtgccaggcccacggcttgacccctcagcaggtggtggccatcgccagcaatggcggcggcaggccggcgctggagagcattgttgcccagttatctcgccctgatccggcgttggccgcgttgaccaacgaccacctcgtcgccttggcctgcctcggcgggcgtcctgcgctggatgcagtgaaaaagggattgggggatcctatcagccgttcccagctggtgaagtccgagctggaggagaagaaatccgagttgaggcacaagctgaagtacgtgccccacgagtacatcgagctgatcgagatcgcccggaacagcacccaggaccgtatcctggagatgaaggtgatggagttcttcatgaaggtgtacggctacaggggcaagcacctgggcggctccaggaagcccgacggcgccatctacaccgtgggctcccccatcgactacggcgtgatcgtggacaccaaggcctactccggcggctacaacctgcccatcggccaggccgacgaaatgcagaggtacgtggaggagaaccagaccaggaacaagcacatcaaccccaacgagtggtggaaggtgtacccctccagcgtgaccgagttcaagttcctgttcgtgtccggccacttcaagggcaactacaaggcccagctgaccaggctgaaccacatcaccaactgcaacggcgccgtgctgtccgtggaggagctcctgatcggcggcgagatgatcaaggccggcaccctgaccctggaggaggtgaggaggaagttcaacaacggcgagatcaacttcgcggccgactgataa

SEQ ID NO: 72 - DNA, 2832 bp, Artificial Sequence
  TALE-nuclease sequence
atgggcgatcctaaaaagaaacgtaaggtcatcgataaggagaccgccgctgccaagttcgagagacagcacatggacagcatcgatatcgccgatctacgcacgctcggctacagccagcagcaacaggagaagatcaaaccgaaggttcgttcgacagtggcgcagcaccacgaggcactggtcggccacgggtttacacacgcgcacatcgttgcgttaagccaacacccggcagcgttagggaccgtcgctgtcaagtatcaggacatgatcgcagcgttgccagaggcgacacacgaagcgatcgttggcgtcggcaaacagtggtccggcgcacgcgctctggaggccttgctcacggtggcgggagagttgagaggtccaccgttacagttggacacaggccaacttctcaagattgcaaaacgtggcggcgtgaccgcagtggaggcagtgcatgcatggcgcaatgcactgacgggtgccccgctcaacttgaccccccagcaggtggtggccatcgccagcaataatggtggcaagcaggcgctggagacggtccagcggctgttgccggtgctgtgccaggcccacggcttgaccccccagcaggtggtggccatcgccagcaatggcggtggcaagcaggcgctggagacggtccagcggctgttgccggtgctgtgccaggcccacggcttgaccccccagcaggtggtggccatcgccagcaataatggtggcaagcaggcgctggagacggtccagcggctgttgccggtgctgtgccaggcccacggcttgaccccccagcaggtggtggccatcgccagcaataatggtggcaagcaggcgctggagacggtccagcggctgttgccggtgctgtgccaggcccacggcttgaccccggagcaggtggtggccatcgccagccacgatggcggcaagcaggcgctggagacggtccagcggctgttgccggtgctgtgccaggcccacggcttgaccccggagcaggtggtggccatcgccagccacgatggcggcaagcaggcgctggagacggtccagcggctgttgccggtgctgtgccaggcccacggcttgaccccccagcaggtggtggccatcgccagcaatggcggtggcaagcaggcgctggagacggtccagcggctgttgccggtgctgtgccaggcccacggcttgaccccccagcaggtggtggccatcgccagcaatggcggtggcaagcaggcgctggagacggtccagcggctgttgccggtgctgtgccaggcccacggcttgaccccccagcaggtggtggccatcgccagcaatggcggtggcaagcaggcgctggagacggtccagcggctgttgccggtgctgtgccaggcccacggcttgaccccccagcaggtggtggccatcgccagcaatggcggtggcaagcaggcgctggagacggtccagcggctgttgccggtgctgtgccaggcccacggcttgaccccccagcaggtggtggccatcgccagcaataatggtggcaagcaggcgctggagacggtccagcggctgttgccggtgctgtgccaggcccacggcttgaccccccagcaggtggtggccatcgccagcaataatggtggcaagcaggcgctggagacggtccagcggctgttgccggtgctgtgccaggcccacggcttgaccccccagcaggtggtggccatcgccagcaataatggtggcaagcaggcgctggagacggtccagcggctgttgccggtgctgtgccaggcccacggcttgaccccccagcaggtggtggccatcgccagcaatggcggtggcaagcaggcgctggagacggtccagcggctgttgccggtgctgtgccaggcccacggcttgaccccccagcaggtggtggccatcgccagcaataatggtggcaagcaggcgctggagacggtccagcggctgttgccggtgctgtgccaggcccacggcttgacccctcagcaggtggtggccatcgccagcaatggcggcggcaggccggcgctggagagcattgttgcccagttatctcgccctgatccggcgttggccgcgttgaccaacgaccacctcgtcgccttggcctgcctcggcgggcgtcctgcgctggatgcagtgaaaaagggattgggggatcctatcagccgttcccagctggtgaagtccgagctggaggagaagaaatccgagttgaggcacaagctgaagtacgtgccccacgagtacatcgagctgatcgagatcgcccggaacagcacccaggaccgtatcctggagatgaaggtgatggagttcttcatgaaggtgtacggctacaggggcaagcacctgggcggctccaggaagcccgacggcgccatctacaccgtgggctcccccatcgactacggcgtgatcgtggacaccaaggcctactccggcggctacaacctgcccatcggccaggccgacgaaatgcagaggtacgtggaggagaaccagaccaggaacaagcacatcaaccccaacgagtggtggaaggtgtacccctccagcgtgaccgagttcaagttcctgttcgtgtccggccacttcaagggcaactacaaggcccagctgaccaggctgaaccacatcaccaactgcaacggcgccgtgctgtccgtggaggagctcctgatcggcggcgagatgatcaaggccggcaccctgaccctggaggaggtgaggaggaagttcaacaacggcgagatcaacttcgcggccgactgataa

SEQ ID NO: 73 - DNA, 2814 bp, Artificial Sequence
  TALE-nuclease sequence
atgggcgatcctaaaaagaaacgtaaggtcatcgattacccatacgatgttccagattacgctatcgatatcgccgatctacgcacgctcggctacagccagcagcaacaggagaagatcaaaccgaaggttcgttcgacagtggcgcagcaccacgaggcactggtcggccacgggtttacacacgcgcacatcgttgcgttaagccaacacccggcagcgttagggaccgtcgctgtcaagtatcaggacatgatcgcagcgttgccagaggcgacacacgaagcgatcgttggcgtcggcaaacagtggtccggcgcacgcgctctggaggccttgctcacggtggcgggagagttgagaggtccaccgttacagttggacacaggccaacttctcaagattgcaaaacgtggcggcgtgaccgcagtggaggcagtgcatgcatggcgcaatgcactgacgggtgccccgctcaacttgaccccggagcaggtggtggccatcgccagccacgatggcggcaagcaggcgctggagacggtccagcggctgttgccggtgctgtgccaggcccacggcttgaccccggagcaggtggtggccatcgccagccacgatggcggcaagcaggcgctggagacggtccagcggctgttgccggtgctgtgccaggcccacggcttgaccccggagcaggtggtggccatcgccagccacgatggcggcaagcaggcgctggagacggtccagcggctgttgccggtgctgtgccaggcccacggcttgaccccggagcaggtggtggccatcgccagcaatattggtggcaagcaggcgctggagacggtgcaggcgctgttgccggtgctgtgccaggcccacggcttgaccccggagcaggtggtggccatcgccagccacgatggcggcaagcaggcgctggagacggtccagcggctgttgccggtgctgtgccaggcccacggcttgaccccggagcaggtggtggccatcgccagccacgatggcggcaagcaggcgctggagacggtccagcggctgttgccggtgctgtgccaggcccacggcttgaccccggagcaggtggtggccatcgccagccacgatggcggcaagcaggcgctggagacggtccagcggctgttgccggtgctgtgccaggcccacggcttgaccccccagcaggtggtggccatcgccagcaataatggtggcaagcaggcgctggagacggtccagcggctgttgccggtgctgtgccaggcccacggcttgaccccggagcaggtggtggccatcgccagcaatattggtggcaagcaggcgctggagacggtgcaggcgctgttgccggtgctgtgccaggcccacggcttgaccccccagcaggtggtggccatcgccagcaataatggtggcaagcaggcgctggagacggtccagcggctgttgccggtgctgtgccaggcccacggcttgaccccccagcaggtggtggccatcgccagcaataatggtggcaagcaggcgctggagacggtccagcggctgttgccggtgctgtgccaggcccacggcttgaccccccagcaggtggtggccatcgccagcaatggcggtggcaagcaggcgctggagacggtccagcggctgttgccggtgctgtgccaggcccacggcttgaccccggagcaggtggtggccatcgccagccacgatggcggcaagcaggcgctggagacggtccagcggctgttgccggtgctgtgccaggcccacggcttgaccccccagcaggtggtggccatcgccagcaataatggtggcaagcaggcgctggagacggtccagcggctgttgccggtgctgtgccaggcccacggcttgaccccggagcaggtggtggccatcgccagccacgatggcggcaagcaggcgctggagacggtccagcggctgttgccggtgctgtgccaggcccacggcttgacccctcagcaggtggtggccatcgccagcaatggcggcggcaggccggcgctggagagcattgttgcccagttatctcgccctgatccggcgttggccgcgttgaccaacgaccacctcgtcgccttggcctgcctcggcgggcgtcctgcgctggatgcagtgaaaaagggattgggggatcctatcagccgttcccagctggtgaagtccgagctggaggagaagaaatccgagttgaggcacaagctgaagtacgtgccccacgagtacatcgagctgatcgagatcgcccggaacagcacccaggaccgtatcctggagatgaaggtgatggagttcttcatgaaggtgtacggctacaggggcaagcacctgggcggctccaggaagcccgacggcgccatctacaccgtgggctcccccatcgactacggcgtgatcgtggacaccaaggcctactccggcggctacaacctgcccatcggccaggccgacgaaatgcagaggtacgtggaggagaaccagaccaggaacaagcacatcaaccccaacgagtggtggaaggtgtacccctccagcgtgaccgagttcaagttcctgttcgtgtccggccacttcaagggcaactacaaggcccagctgaccaggctgaaccacatcaccaactgcaacggcgccgtgctgtccgtggaggagctcctgatcggcggcgagatgatcaaggccggcaccctgaccctggaggaggtgaggaggaagttcaacaacggcgagatcaacttcgcggccgactgataa

SEQ ID NO: 74 - DNA, 2832 bp, Artificial Sequence
  TALE-nuclease sequence
atgggcgatcctaaaaagaaacgtaaggtcatcgataaggagaccgccgctgccaagttcgagagacagcacatggacagcatcgatatcgccgatctacgcacgctcggctacagccagcagcaacaggagaagatcaaaccgaaggttcgttcgacagtggcgcagcaccacgaggcactggtcggccacgggtttacacacgcgcacatcgttgcgttaagccaacacccggcagcgttagggaccgtcgctgtcaagtatcaggacatgatcgcagcgttgccagaggcgacacacgaagcgatcgttggcgtcggcaaacagtggtccggcgcacgcgctctggaggccttgctcacggtggcgggagagttgagaggtccaccgttacagttggacacaggccaacttctcaagattgcaaaacgtggcggcgtgaccgcagtggaggcagtgcatgcatggcgcaatgcactgacgggtgccccgctcaacttgaccccccagcaggtggtggccatcgccagcaataatggtggcaagcaggcgctggagacggtccagcggctgttgccggtgctgtgccaggcccacggcttgaccccccagcaggtggtggccatcgccagcaataatggtggcaagcaggcgctggagacggtccagcggctgttgccggtgctgtgccaggcccacggcttgaccccccagcaggtggtggccatcgccagcaataatggtggcaagcaggcgctggagacggtccagcggctgttgccggtgctgtgccaggcccacggcttgaccccggagcaggtggtggccatcgccagcaatattggtggcaagcaggcgctggagacggtgcaggcgctgttgccggtgctgtgccaggcccacggcttgaccccccagcaggtggtggccatcgccagcaataatggtggcaagcaggcgctggagacggtccagcggctgttgccggtgctgtgccaggcccacggcttgaccccggagcaggtggtggccatcgccagcaatattggtggcaagcaggcgctggagacggtgcaggcgctgttgccggtgctgtgccaggcccacggcttgaccccccagcaggtggtggccatcgccagcaatggcggtggcaagcaggcgctggagacggtccagcggctgttgccggtgctgtgccaggcccacggcttgaccccggagcaggtggtggccatcgccagccacgatggcggcaagcaggcgctggagacggtccagcggctgttgccggtgctgtgccaggcccacggcttgaccccccagcaggtggtggccatcgccagcaatggcggtggcaagcaggcgctggagacggtccagcggctgttgccggtgctgtgccaggcccacggcttgaccccggagcaggtggtggccatcgccagccacgatggcggcaagcaggcgctggagacggtccagcggctgttgccggtgctgtgccaggcccacggcttgaccccccagcaggtggtggccatcgccagcaatggcggtggcaagcaggcgctggagacggtccagcggctgttgccggtgctgtgccaggcccacggcttgaccccccagcaggtggtggccatcgccagcaataatggtggcaagcaggcgctggagacggtccagcggctgttgccggtgctgtgccaggcccacggcttgaccccggagcaggtggtggccatcgccagccacgatggcggcaagcaggcgctggagacggtccagcggctgttgccggtgctgtgccaggcccacggcttgaccccccagcaggtggtggccatcgccagcaatggcggtggcaagcaggcgctggagacggtccagcggctgttgccggtgctgtgccaggcccacggcttgaccccccagcaggtggtggccatcgccagcaatggcggtggcaagcaggcgctggagacggtccagcggctgttgccggtgctgtgccaggcccacggcttgacccctcagcaggtggtggccatcgccagcaatggcggcggcaggccggcgctggagagcattgttgcccagttatctcgccctgatccggcgttggccgcgttgaccaacgaccacctcgtcgccttggcctgcctcggcgggcgtcctgcgctggatgcagtgaaaaagggattgggggatcctatcagccgttcccagctggtgaagtccgagctggaggagaagaaatccgagttgaggcacaagctgaagtacgtgccccacgagtacatcgagctgatcgagatcgcccggaacagcacccaggaccgtatcctggagatgaaggtgatggagttcttcatgaaggtgtacggctacaggggcaagcacctgggcggctccaggaagcccgacggcgccatctacaccgtgggctcccccatcgactacggcgtgatcgtggacaccaaggcctactccggcggctacaacctgcccatcggccaggccgacgaaatgcagaggtacgtggaggagaaccagaccaggaacaagcacatcaaccccaacgagtggtggaaggtgtacccctccagcgtgaccgagttcaagttcctgttcgtgtccggccacttcaagggcaactacaaggcccagctgaccaggctgaaccacatcaccaactgcaacggcgccgtgctgtccgtggaggagctcctgatcggcggcgagatgatcaaggccggcaccctgaccctggaggaggtgaggaggaagttcaacaacggcgagatcaacttcgcggccgactgataa

SEQ ID NO: 75 - DNA, 21 bp, Artificial Sequence
  PCR primer
atcactggcatctggactcca

SEQ ID NO: 76 - DNA, 22 bp, Artificial Sequence
  PCR primer
agagcccctaccagaaccagac

SEQ ID NO: 77 - DNA, 22 bp, Artificial Sequence
  PCR primer
ggacctagtaacataattgtgc

SEQ ID NO: 78 - DNA, 20 bp, Artificial Sequence
  PCR primer
cctcatgtctagcacagttt

SEQ ID NO: 79 - DNA, 21 bp, Artificial Sequence
  PCR primer
accagctcagctccacgtggt

SEQ ID NO: 80 - DNA, 58 bp, Homo sapiens
tctcgctccgtggccttagctgtgctcgcgctactctctctttctggcctggaggcta

SEQ ID NO: 81 - DNA, 2814 bp, Artificial Sequence
  Beta2M T01- TALEN - LEFT
atgggcgatcctaaaaagaaacgtaaggtcatcgattacccatacgatgttccagattacgctatcgatatcgccgatctacgcacgctcggctacagccagcagcaacaggagaagatcaaaccgaaggttcgttcgacagtggcgcagcaccacgaggcactggtcggccacgggtttacacacgcgcacatcgttgcgttaagccaacacccggcagcgttagggaccgtcgctgtcaagtatcaggacatgatcgcagcgttgccagaggcgacacacgaagcgatcgttggcgtcggcaaacagtggtccggcgcacgcgctctggaggccttgctcacggtggcgggagagttgagaggtccaccgttacagttggacacaggccaacttctcaagattgcaaaacgtggcggcgtgaccgcagtggaggcagtgcatgcatggcgcaatgcactgacgggtgccccgctcaacttgaccccccagcaggtggtggccatcgccagcaataatggtggcaagcaggcgctggagacggtccagcggctgttgccggtgctgtgccaggcccacggcttgaccccccagcaggtggtggccatcgccagcaataatggtggcaagcaggcgctggagacggtccagcggctgttgccggtgctgtgccaggcccacggcttgaccccggagcaggtggtggccatcgccagccacgatggcggcaagcaggcgctggagacggtccagcggctgttgccggtgctgtgccaggcccacggcttgaccccggagcaggtggtggccatcgccagccacgatggcggcaagcaggcgctggagacggtccagcggctgttgccggtgctgtgccaggcccacggcttgaccccccagcaggtggtggccatcgccagcaatggcggtggcaagcaggcgctggagacggtccagcggctgttgccggtgctgtgccaggcccacggcttgaccccccagcaggtggtggccatcgccagcaatggcggtggcaagcaggcgctggagacggtccagcggctgttgccggtgctgtgccaggcccacggcttgaccccggagcaggtggtggccatcgccagcaatattggtggcaagcaggcgctggagacggtgcaggcgctgttgccggtgctgtgccaggcccacggcttgaccccccagcaggtggtggccatcgccagcaataatggtggcaagcaggcgctggagacggtccagcggctgttgccggtgctgtgccaggcccacggcttgaccccggagcaggtggtggccatcgccagccacgatggcggcaagcaggcgctggagacggtccagcggctgttgccggtgctgtgccaggcccacggcttgaccccccagcaggtggtggccatcgccagcaatggcggtggcaagcaggcgctggagacggtccagcggctgttgccggtgctgtgccaggcccacggcttgaccccccagcaggtggtggccatcgccagcaataatggtggcaagcaggcgctggagacggtccagcggctgttgccggtgctgtgccaggcccacggcttgaccccccagcaggtggtggccatcgccagcaatggcggtggcaagcaggcgctggagacggtccagcggctgttgccggtgctgtgccaggcccacggcttgaccccccagcaggtggtggccatcgccagcaataatggtggcaagcaggcgctggagacggtccagcggctgttgccggtgctgtgccaggcccacggcttgaccccggagcaggtggtggccatcgccagccacgatggcggcaagcaggcgctggagacggtccagcggctgttgccggtgctgtgccaggcccacggcttgaccccccagcaggtggtggccatcgccagcaatggcggtggcaagcaggcgctggagacggtccagcggctgttgccggtgctgtgccaggcccacggcttgacccctcagcaggtggtggccatcgccagcaatggcggcggcaggccggcgctggagagcattgttgcccagttatctcgccctgatccggcgttggccgcgttgaccaacgaccacctcgtcgccttggcctgcctcggcgggcgtcctgcgctggatgcagtgaaaaagggattgggggatcctatcagccgttcccagctggtgaagtccgagctggaggagaagaaatccgagttgaggcacaagctgaagtacgtgccccacgagtacatcgagctgatcgagatcgcccggaacagcacccaggaccgtatcctggagatgaaggtgatggagttcttcatgaaggtgtacggctacaggggcaagcacctgggcggctccaggaagcccgacggcgccatctacaccgtgggctcccccatcgactacggcgtgatcgtggacaccaaggcctactccggcggctacaacctgcccatcggccaggccgacgaaatgcagaggtacgtggaggagaaccagaccaggaacaagcacatcaaccccaacgagtggtggaaggtgtacccctccagcgtgaccgagttcaagttcctgttcgtgtccggccacttcaagggcaactacaaggcccagctgaccaggctgaaccacatcaccaactgcaacggcgccgtgctgtccgtggaggagctcctgatcggcggcgagatgatcaaggccggcaccctgaccctggaggaggtgaggaggaagttcaacaacggcgagatcaacttcgcggccgactgataa

SEQ ID NO: 82 - DNA, 2832 bp, Artificial Sequence
  Beta2M T01 TALEN -RIGHT
atgggcgatcctaaaaagaaacgtaaggtcatcgataaggagaccgccgctgccaagttcgagagacagcacatggacagcatcgatatcgccgatctacgcacgctcggctacagccagcagcaacaggagaagatcaaaccgaaggttcgttcgacagtggcgcagcaccacgaggcactggtcggccacgggtttacacacgcgcacatcgttgcgttaagccaacacccggcagcgttagggaccgtcgctgtcaagtatcaggacatgatcgcagcgttgccagaggcgacacacgaagcgatcgttggcgtcggcaaacagtggtccggcgcacgcgctctggaggccttgctcacggtggcgggagagttgagaggtccaccgttacagttggacacaggccaacttctcaagattgcaaaacgtggcggcgtgaccgcagtggaggcagtgcatgcatggcgcaatgcactgacgggtgccccgctcaacttgaccccggagcaggtggtggccatcgccagcaatattggtggcaagcaggcgctggagacggtgcaggcgctgttgccggtgctgtgccaggcccacggcttgaccccccagcaggtggtggccatcgccagcaataatggtggcaagcaggcgctggagacggtccagcggctgttgccggtgctgtgccaggcccacggcttgaccccggagcaggtggtggccatcgccagccacgatggcggcaagcaggcgctggagacggtccagcggctgttgccggtgctgtgccaggcccacggcttgaccccggagcaggtggtggccatcgccagccacgatggcggcaagcaggcgctggagacggtccagcggctgttgccggtgctgtgccaggcccacggcttgaccccccagcaggtggtggccatcgccagcaatggcggtggcaagcaggcgctggagacggtccagcggctgttgccggtgctgtgccaggcccacggcttgaccccggagcaggtggtggccatcgccagccacgatggcggcaagcaggcgctggagacggtccagcggctgttgccggtgctgtgccaggcccacggcttgaccccggagcaggtggtggccatcgccagccacgatggcggcaagcaggcgctggagacggtccagcggctgttgccggtgctgtgccaggcccacggcttgaccccggagcaggtggtggccatcgccagcaatattggtggcaagcaggcgctggagacggtgcaggcgctgttgccggtgctgtgccaggcccacggcttgaccccccagcaggtggtggccatcgccagcaataatggtggcaagcaggcgctggagacggtccagcggctgttgccggtgctgtgccaggcccacggcttgaccccccagcaggtggtggccatcgccagcaataatggtggcaagcaggcgctggagacggtccagcggctgttgccggtgctgtgccaggcccacggcttgaccccggagcaggtggtggccatcgccagccacgatggcggcaagcaggcgctggagacggtccagcggctgttgccggtgctgtgccaggcccacggcttgaccccggagcaggtggtggccatcgccagccacgatggcggcaagcaggcgctggagacggtccagcggctgttgccggtgctgtgccaggcccacggcttgaccccggagcaggtggtggccatcgccagcaatattggtggcaagcaggcgctggagacggtgcaggcgctgttgccggtgctgtgccaggcccacggcttgaccccccagcaggtggtggccatcgccagcaataatggtggcaagcaggcgctggagacggtccagcggctgttgccggtgctgtgccaggcccacggcttgaccccggagcaggtggtggccatcgccagcaatattggtggcaagcaggcgctggagacggtgcaggcgctgttgccggtgctgtgccaggcccacggcttgacccctcagcaggtggtggccatcgccagcaatggcggcggcaggccggcgctggagagcattgttgcccagttatctcgccctgatccggcgttggccgcgttgaccaacgaccacctcgtcgccttggcctgcctcggcgggcgtcctgcgctggatgcagtgaaaaagggattgggggatcctatcagccgttcccagctggtgaagtccgagctggaggagaagaaatccgagttgaggcacaagctgaagtacgtgccccacgagtacatcgagctgatcgagatcgcccggaacagcacccaggaccgtatcctggagatgaaggtgatggagttcttcatgaaggtgtacggctacaggggcaagcacctgggcggctccaggaagcccgacggcgccatctacaccgtgggctcccccatcgactacggcgtgatcgtggacaccaaggcctactccggcggctacaacctgcccatcggccaggccgacgaaatgcagaggtacgtggaggagaaccagaccaggaacaagcacatcaaccccaacgagtggtggaaggtgtacccctccagcgtgaccgagttcaagttcctgttcgtgtccggccacttcaagggcaactacaaggcccagctgaccaggctgaaccacatcaccaactgcaacggcgccgtgctgtccgtggaggagctcctgatcggcggcgagatgatcaaggccggcaccctgaccctggaggaggtgaggaggaagttcaacaacggcgagatcaacttcgcggccgactgataa

SEQ ID NO: 83 - DNA, 50 bp, Artificial Sequence
  B2M T02- TALEN targeting sequence
tccaaagattcaggtttactcacgtcatccagcagagaatggaaagtcaa

SEQ ID NO: 84 - DNA, 2814 bp, Artificial Sequence; identical to SEQ ID NO: 67
  Beta2M T02-TALEN - LEFT

SEQ ID NO: 85 - DNA, 2832 bp, Artificial Sequence; identical to SEQ ID NO: 68
  Beta2M T02-TALEN  RIGHT

SEQ ID NO: 86 - DNA, 47 bp, Artificial Sequence
  B2M T03- TALEN targeting sequence
ttagctgtgctcgcgctactctctctttctggcctggaggctatcca

SEQ ID NO: 87 - DNA, 2814 bp, Artificial Sequence
  Beta2M T03-TALEN - LEFT
atgggcgatcctaaaaagaaacgtaaggtcatcgattacccatacgatgttccagattacgctatcgatatcgccgatctacgcacgctcggctacagccagcagcaacaggagaagatcaaaccgaaggttcgttcgacagtggcgcagcaccacgaggcactggtcggccacgggtttacacacgcgcacatcgttgcgttaagccaacacccggcagcgttagggaccgtcgctgtcaagtatcaggacatgatcgcagcgttgccagaggcgacacacgaagcgatcgttggcgtcggcaaacagtggtccggcgcacgcgctctggaggccttgctcacggtggcgggagagttgagaggtccaccgttacagttggacacaggccaacttctcaagattgcaaaacgtggcggcgtgaccgcagtggaggcagtgcatgcatggcgcaatgcactgacgggtgccccgctcaacttgaccccggagcaggtggtggccatcgccagcaatattggtggcaagcaggcgctggagacggtgcaggcgctgttgccggtgctgtgccaggcccacggcttgaccccccagcaggtggtggccatcgccagcaataatggtggcaagcaggcgctggagacggtccagcggctgttgccggtgctgtgccaggcccacggcttgaccccggagcaggtggtggccatcgccagccacgatggcggcaagcaggcgctggagacggtccagcggctgttgccggtgctgtgccaggcccacggcttgaccccccagcaggtggtggccatcgccagcaatggcggtggcaagcaggcgctggagacggtccagcggctgttgccggtgctgtgccaggcccacggcttgaccccccagcaggtggtggccatcgccagcaataatggtggcaagcaggcgctggagacggtccagcggctgttgccggtgctgtgccaggcccacggcttgaccccccagcaggtggtggccatcgccagcaatggcggtggcaagcaggcgctggagacggtccagcggctgttgccggtgctgtgccaggcccacggcttgaccccccagcaggtggtggccatcgccagcaataatggtggcaagcaggcgctggagacggtccagcggctgttgccggtgctgtgccaggcccacggcttgaccccggagcaggtggtggccatcgccagccacgatggcggcaagcaggcgctggagacggtccagcggctgttgccggtgctgtgccaggcccacggcttgaccccccagcaggtggtggccatcgccagcaatggcggtggcaagcaggcgctggagacggtccagcggctgttgccggtgctgtgccaggcccacggcttgaccccggagcaggtggtggccatcgccagccacgatggcggcaagcaggcgctggagacggtccagcggctgttgccggtgctgtgccaggcccacggcttgaccccccagcaggtggtggccatcgccagcaataatggtggcaagcaggcgctggagacggtccagcggctgttgccggtgctgtgccaggcccacggcttgaccccggagcaggtggtggccatcgccagccacgatggcggcaagcaggcgctggagacggtccagcggctgttgccggtgctgtgccaggcccacggcttgaccccccagcaggtggtggccatcgccagcaataatggtggcaagcaggcgctggagacggtccagcggctgttgccggtgctgtgccaggcccacggcttgaccccggagcaggtggtggccatcgccagccacgatggcggcaagcaggcgctggagacggtccagcggctgttgccggtgctgtgccaggcccacggcttgaccccccagcaggtggtggccatcgccagcaatggcggtggcaagcaggcgctggagacggtccagcggctgttgccggtgctgtgccaggcccacggcttgacccctcagcaggtggtggccatcgccagcaatggcggcggcaggccggcgctggagagcattgttgcccagttatctcgccctgatccggcgttggccgcgttgaccaacgaccacctcgtcgccttggcctgcctcggcgggcgtcctgcgctggatgcagtgaaaaagggattgggggatcctatcagccgttcccagctggtgaagtccgagctggaggagaagaaatccgagttgaggcacaagctgaagtacgtgccccacgagtacatcgagctgatcgagatcgcccggaacagcacccaggaccgtatcctggagatgaaggtgatggagttcttcatgaaggtgtacggctacaggggcaagcacctgggcggctccaggaagcccgacggcgccatctacaccgtgggctcccccatcgactacggcgtgatcgtggacaccaaggcctactccggcggctacaacctgcccatcggccaggccgacgaaatgcagaggtacgtggaggagaaccagaccaggaacaagcacatcaaccccaacgagtggtggaaggtgtacccctccagcgtgaccgagttcaagttcctgttcgtgtccggccacttcaagggcaactacaaggcccagctgaccaggctgaaccacatcaccaactgcaacggcgccgtgctgtccgtggaggagctcctgatcggcggcgagatgatcaaggccggcaccctgaccctggaggaggtgaggaggaagttcaacaacggcgagatcaacttcgcggccgactgataa

SEQ ID NO: 88 - DNA, 2832 bp, Artificial Sequence
  Beta2M T03-TALEN -RIGHT
atgggcgatcctaaaaagaaacgtaaggtcatcgataaggagaccgccgctgccaagttcgagagacagcacatggacagcatcgatatcgccgatctacgcacgctcggctacagccagcagcaacaggagaagatcaaaccgaaggttcgttcgacagtggcgcagcaccacgaggcactggtcggccacgggtttacacacgcgcacatcgttgcgttaagccaacacccggcagcgttagggaccgtcgctgtcaagtatcaggacatgatcgcagcgttgccagaggcgacacacgaagcgatcgttggcgtcggcaaacagtggtccggcgcacgcgctctggaggccttgctcacggtggcgggagagttgagaggtccaccgttacagttggacacaggccaacttctcaagattgcaaaacgtggcggcgtgaccgcagtggaggcagtgcatgcatggcgcaatgcactgacgggtgccccgctcaacttgaccccccagcaggtggtggccatcgccagcaataatggtggcaagcaggcgctggagacggtccagcggctgttgccggtgctgtgccaggcccacggcttgaccccccagcaggtggtggccatcgccagcaataatggtggcaagcaggcgctggagacggtccagcggctgttgccggtgctgtgccaggcccacggcttgaccccggagcaggtggtggccatcgccagcaatattggtggcaagcaggcgctggagacggtgcaggcgctgttgccggtgctgtgccaggcccacggcttgaccccccagcaggtggtggccatcgccagcaatggcggtggcaagcaggcgctggagacggtccagcggctgttgccggtgctgtgccaggcccacggcttgaccccggagcaggtggtggccatcgccagcaatattggtggcaagcaggcgctggagacggtgcaggcgctgttgccggtgctgtgccaggcccacggcttgaccccccagcaggtggtggccatcgccagcaataatggtggcaagcaggcgctggagacggtccagcggctgttgccggtgctgtgccaggcccacggcttgaccccggagcaggtggtggccatcgccagccacgatggcggcaagcaggcgctggagacggtccagcggctgttgccggtgctgtgccaggcccacggcttgaccccggagcaggtggtggccatcgccagccacgatggcggcaagcaggcgctggagacggtccagcggctgttgccggtgctgtgccaggcccacggcttgaccccccagcaggtggtggccatcgccagcaatggcggtggcaagcaggcgctggagacggtccagcggctgttgccggtgctgtgccaggcccacggcttgaccccggagcaggtggtggccatcgccagccacgatggcggcaagcaggcgctggagacggtccagcggctgttgccggtgctgtgccaggcccacggcttgaccccggagcaggtggtggccatcgccagccacgatggcggcaagcaggcgctggagacggtccagcggctgttgccggtgctgtgccaggcccacggcttgaccccggagcaggtggtggccatcgccagcaatattggtggcaagcaggcgctggagacggtgcaggcgctgttgccggtgctgtgccaggcccacggcttgaccccccagcaggtggtggccatcgccagcaataatggtggcaagcaggcgctggagacggtccagcggctgttgccggtgctgtgccaggcccacggcttgaccccccagcaggtggtggccatcgccagcaataatggtggcaagcaggcgctggagacggtccagcggctgttgccggtgctgtgccaggcccacggcttgaccccggagcaggtggtggccatcgccagccacgatggcggcaagcaggcgctggagacggtccagcggctgttgccggtgctgtgccaggcccacggcttgacccctcagcaggtggtggccatcgccagcaatggcggcggcaggccggcgctggagagcattgttgcccagttatctcgccctgatccggcgttggccgcgttgaccaacgaccacctcgtcgccttggcctgcctcggcgggcgtcctgcgctggatgcagtgaaaaagggattgggggatcctatcagccgttcccagctggtgaagtccgagctggaggagaagaaatccgagttgaggcacaagctgaagtacgtgccccacgagtacatcgagctgatcgagatcgcccggaacagcacccaggaccgtatcctggagatgaaggtgatggagttcttcatgaaggtgtacggctacaggggcaagcacctgggcggctccaggaagcccgacggcgccatctacaccgtgggctcccccatcgactacggcgtgatcgtggacaccaaggcctactccggcggctacaacctgcccatcggccaggccgacgaaatgcagaggtacgtggaggagaaccagaccaggaacaagcacatcaaccccaacgagtggtggaaggtgtacccctccagcgtgaccgagttcaagttcctgttcgtgtccggccacttcaagggcaactacaaggcccagctgaccaggctgaaccacatcaccaactgcaacggcgccgtgctgtccgtggaggagctcctgatcggcggcgagatgatcaaggccggcaccctgaccctggaggaggtgaggaggaagttcaacaacggcgagatcaacttcgcggccgactgataa

SEQ ID NO: 89 - protein, 526 aa, Artificial Sequence [sequence omitted]

SEQ ID NO: 90 - protein, 310 aa, Artificial Sequence
  SP-MICAed
MGGVLLTQRTLLSLVLALLFPSMASMEPHSLRYNLTVLSWDGSVQSGFLTEVHLDGQPFLRCDRQKCRAKPQGQWAEDVLGNKTWDRETRDLTGNGKDLRMTLAHIKDQKEGLHSLQEIRVCEIHEDNSTRSSQHFYYDGELFLSQNLETKEWTMPQSSRAQTLAMNVRNFLKEDAMKTKTHYHAMHADCLQELRRYLKSGVVLRRTVPPMVNVTRSEASEGNITVTCRASGFYPWNITLSWRQDGVSLSHDTQQWGDVLPDGNGTYQTWVATRICQGEEQRFTCYMEHSGNHSTHPVPSGKVLVLQSHW

SEQ ID NO: 91 - protein, 313 aa, Artificial Sequence
  SP-MICBed
MGGVLLTQRTLLSLVLALLFPSMASMAEPHSLRYNLMVLSQDESVQSGFLAEGHLDGQPFLRYDRQKRRAKPQGQWAEDVLGAKTWDTETEDLTENGQDLRRTLTHIKDQKGGLHSLQEIRVCEIHEDSSTRGSRHFYYDGELFLSQNLETQESTVPQSSRAQTLAMNVTNFWKEDAMKTKTHYRAMQADCLQKLQRYLKSGVAIRRTVPPMVNVTCSEVSEGNITVTCRASSFYPRNITLTWRQDGVSLSHNTQQWGDVLPDGNGTYQTWVATRIRQGEEQRFTCYMEHSGNHGTHPVPSGKVLVLQSQRTD

SEQ ID NO: 92 - protein, 209 aa, Artificial Sequence
  SP-ULBP1ed
MGGVLLTQRTLLSLVLALLFPSMASMGWVDTHCLCYDFIITPKSRPEPQWCEVQGLVDERPFLHYDCVNHKAKAFASLGKKVNVTKTWEEQTETLRDVVDFLKGQLLDIQVENLIPIEPLTLQARMSCEHEAHGHGRGSWQFLFNGQKFLLFDSNNRKWTALHPGAKKMTEKWEKNRDVTMFFQKISLGDCKMWLEEFLMYWEQMLDPT

SEQ ID NO: 93 - protein, 211 aa, Artificial Sequence
  SP-ULBP2ed
MGGVLLTQRTLLSLVLALLFPSMASMGRADPHSLCYDITVIPKFRPGPRWCAVQGQVDEKTFLHYDCGNKTVTPVSPLGKKLNVTTAWKAQNPVLREVVDILTEQLRDIQLENYTPKEPLTLQARMSCEQKAEGHSSGSWQFSFDGQIFLLFDSEKRMWTTVHPGARKMKEKWENDKVVAMSFHYFSMGDCIGWLEDFLMGMDSTLEPSAG

SEQ ID NO: 94 - protein, 206 aa, Artificial Sequence
  SP-ULBP3ed
MGGVLLTQRTLLSLVLALLFPSMASMDAHSLWYNFTIIHLPRHGQQWCEVQSQVDQKNFLSYDCGSDKVLSMGHLEEQLYATDAWGKQLEMLREVGQRLRLELADTELEDFTPSGPLTLQVRMSCECEADGYIRGSWQFSFDGRKFLLFDSNNRKWTVVHAGARRMKEKWEKDSGLTTFFKMVSMRDCKSWLRDFLMHRKKRLEPT

SEQ ID NO: 95 - protein, 221 aa, Artificial Sequence
  SP-N2DL4ed
MGGVLLTQRTLLSLVLALLFPSMASMHSLCFNFTIKSLSRPGQPWCEAQVFLNKNLFLQYNSDNNMVKPLGLLGKKVYATSTWGELTQTLGEVGRDLRMLLCDIKPQIKTSDPSTLQVEMFCQREAERCTGASWQFATNGEKSLLFDAMNMTWTVINHEASKIKETWKKDRGLEKYFRKLSKGDCDHWLREFLGHWEAMPEPTVSPVNASDIHWSSSSLPD

SEQ ID NO: 96 - protein, 224 aa, Artificial Sequence
  SP-RET1Ged
MGGVLLTQRTLLSLVLALLFPSMASMGLADPHSLCYDITVIPKFRPGPRWCAVQGQVDEKTFLHYDCGSKTVTPVSPLGKKLNVTTAWKAQNPVLREVVDILTEQLLDIQLENYIPKEPLTLQARMSCEQKAEGHGSGSWQLSFDGQIFLLFDSENRMWTTVHPGARKMKEKWENDKDMTMSFHYISMGDCTGWLEDFLMGMDSTLEPSAGAPPTMSSGTAQPR

SEQ ID NO: 97 - protein, 211 aa, Artificial Sequence
  SP-RAETILed
MGGVLLTQRTLLSLVLALLFPSMASMRRDDPHSLCYDITVIPKFRPGPRWCAVQGQVDEKTFLHYDCGNKTVTPVSPLGKKLNVTMAWKAQNPVLREVVDILTEQLLDIQLENYTPKEPLTLQARMSCEQKAEGHSSGSWQFSIDGQTFLLFDSEKRMWTTVHPGARKMKEKWENDKDVAMSFHYISMGDCIGWLEDFLMGMDSTLEPSAG